European Patent Application EP 4 741 826 A1, published May 13, 2026. Title: Anti-Nephrin Autoantibody Assay Kits and Detection and Preparation Method Thereof. Applicant: Shenzhen YHLO Biotech Co., Ltd. Application WO. The sequence listing filed with the application follows.

SEQUENCE LISTING (2 sequences)

SEQ ID NO: 1 - protein, 1055 aa, synthetic construct
MGWSCIILFLVATATGVHSQLAIPASVPRGFWALPENLTVVEGASVELRCGVSTPGSAVQWAKDGLLLGPDPRIPGFPRYRLEGDPARGEFHLHIEACDLSDDAEYECQVGRSEMGPELVSPRVILSILVPPKLLLLTPEAGTMVTWVAGQEYVVNCVSGDAKPAPDITILLSGQTISDISANVNEGSQQKLFTVEATARVTPRSSDNRQLLVCEASSPALEAPIKASFTVNVLFPPGPPVIEWPGLDEGHVRAGQSLELPCVARGGNPLATLQWLKNGQPVSTAWGTEHTQAVARSVLVMTVRPEDHGAQLSCEAHNSVSAGTQEHGITLQVTFPPSAIIILGSASQTENKNVTLSCVSKSSRPRVLLRWWLGWRQLLPMEETVMDGLHGGHISMSNLTFLARREDNGLTLTCEAFSEAFTKETFKKSLILNVKYPAQKLWIEGPPEGQKLRAGTRVRLVCLAIGGNPEPSLMWYKDSRTVTESRLPQESRRVHLGSVEKSGSTFSRELVLVTGPSDNQAKFTCKAGQLSASTQLAVQFPPTNVTILANASALRPGDALNLTCVSVSSNPPVNLSWDKEGERLEGVAAPPRRAPFKGSAAARSVLLQVSSRDHGQRVTCRAHSAELRETVSSFYRLNVLYRPEFLGEQVLVVTAVEQGEALLPVSVSANPAPEAFNWTFRGYRLSPAGGPRHRILSSGALHLWNVTRADDGLYQLHCQNSEGTAEARLRLDVHYAPTIRALQDPTEVNVGGSVDIVCTVDANPILPGMFNWERLGEDEEDQSLDDMEKISRGPTGRLRIHHAKLAQAGAYQCIVDNGVAPPARRLLRLVVRFAPQVEHPTPLTKVAAAGDSTSSATLHCRARGVPNIVFTWTKNGVPLDLQDPRYTEHTYHQGGVHSSLLTIANVSAAQDYALFTCTATNALGSDQTNIQLVSISRPDPPSGLKVVSLTPHSVGLEWKPGFDGGLPQRFCIRYEALGTPGFHYVDVVPPQATTFTLTGLQPSTRYRVWLLASNALGDSGLADKGTQLPITTPGLHQPSGEPEDQLPTEPPSGGS

SEQ ID NO: 2 - protein, 1083 aa, synthetic construct
MGWSCIILFLVATATGVHSQLAIPASVPRGFWALPENLTVVEGASVELRCGVSTPGSAVQWAKDGLLLGPDPRIPGFPRYRLEGDPARGEFHLHIEACDLSDDAEYECQVGRSEMGPELVSPRVILSILVPPKLLLLTPEAGTMVTWVAGQEYVVNCVSGDAKPAPDITILLSGQTISDISANVNEGSQQKLFTVEATARVTPRSSDNRQLLVCEASSPALEAPIKASFTVNVLFPPGPPVIEWPGLDEGHVRAGQSLELPCVARGGNPLATLQWLKNGQPVSTAWGTEHTQAVARSVLVMTVRPEDHGAQLSCEAHNSVSAGTQEHGITLQVTFPPSAIIILGSASQTENKNVTLSCVSKSSRPRVLLRWWLGWRQLLPMEETVMDGLHGGHISMSNLTFLARREDNGLTLTCEAFSEAFTKETFKKSLILNVKYPAQKLWIEGPPEGQKLRAGTRVRLVCLAIGGNPEPSLMWYKDSRTVTESRLPQESRRVHLGSVEKSGSTFSRELVLVTGPSDNQAKFTCKAGQLSASTQLAVQFPPTNVTILANASALRPGDALNLTCVSVSSNPPVNLSWDKEGERLEGVAAPPRRAPFKGSAAARSVLLQVSSRDHGQRVTCRAHSAELRETVSSFYRLNVLYRPEFLGEQVLVVTAVEQGEALLPVSVSANPAPEAFNWTFRGYRLSPAGGPRHRILSSGALHLWNVTRADDGLYQLHCQNSEGTAEARLRLDVHYAPTIRALQDPTEVNVGGSVDIVCTVDANPILPGMFNWERLGEDEEDQSLDDMEKISRGPTGRLRIHHAKLAQAGAYQCIVDNGVAPPARRLLRLVVRFAPQVEHPTPLTKVAAAGDSTSSATLHCRARGVPNIVFTWTKNGVPLDLQDPRYTEHTYHQGGVHSSLLTIANVSAAQDYALFTCTATNALGSDQTNIQLVSISRPDPPSGLKVVSLTPHSVGLEWKPGFDGGLPQRFCIRYEALGTPGFHYVDVVPPQATTFTLTGLQPSTRYRVWLLASNALGDSGLADKGTQLPITTPGLHQPSGEPEDQLPTEPPSGGSGLNDIFEAQKIEWHEGGSHHHHHHHHHH